European Patent Application EP 4 574 988 A1, published June 25, 2025. Title: Verfahren zur Herstellung von 2,5-Furandicarbonsäure. Applicant: Annikki GmbH. The sequence listing filed with the application follows.

SEQUENCE LISTING (10 sequences)

SEQ ID NO: 1 - DNA, 1410 bp, Pseudomonas nitroreducens
  source 1..1410: mol_type = genomic DNA
atgtcacgctatgaactgctgatcgatggtcgcctgcaggcggccgagcactacgaccgggtgatcgacccggccagcgaagaaatcgttggcgaagccgcccgcgccagcctggagcaggtcgacgcggcggtggatgccgcacaccgcgccttcccggcctgggccaccgatctcgacgtccgccgccagagcctggcccgagccgccgaacgagtacgcgagaatgcccaggcgctggccgagctgatcacccgcgaacagggtcgcccactgcgctcgaccctggaggaagtggctggcgtcgccgccactttcgagcaccacgcgcagctggagctacccgccgacacccagttgcgcgacgacggcgagcgcctggtgcgcatcacccgcaaaccgctgggggtggtcgccgcgatcaccccgtggaacgtcccgctgatcctgctggtattgaagatcgcgcctgccctgcacgccggcaacaccgtggtggccaagccctcggagcacacgccgctgtctaccctgctgctggcgcgactgctgggcgatgtgttccccgctggcgtgttcaacgtggttgccggtgcgggcgaggttggcgaacacctggtacgtcatccgcgggtgcgccacgtgaccttcaccggcagcgtcgccaccggcaagcgcctgtatgccggcgcgggggacgacctcaagcgtcttaccctggaactgggcggcaacgacgccgcgctggtactggaagacgccgacctcgacgccatcgtcgaaccgctgttctggggcgccttctggaacagcggccaggtgtgctttgcgatcaagcgcctgtacgtgcatgacagcctgttcgaaccgttactggcgaaactcgccgagcgcgcccagcgcacccgcctcggtcatgggctcgacccgcagacggaactggggccgctgaccaacgcacagcaactggaacgggtcatcgccctggtggaagacgccaaggctcacggagcacgcatccgcagcggcggcgtacggcccgacggtcccggctacttctacccgccgaccctggtcagcggcgtggcggccggcgtcgcgctggtggacgaggaacagttcggcccggtgttgccggtgatctccttccgcaacgaagaggacgccattacccaggccaacgccagccactacggcctcggcgcctcggtgtggacccgcgacctggcgcgcggcgaagccatcgccaggcggctggaggcgggcctggcctgggtcaaccagcacggccacatccagcccggcgcgcccaagggcgggcacaagtggagcgggctcggctacgaaggcgggcagcgcggctatgaggccttcagcgagctgcaggtgctgaacatttcgcggcgctaa

SEQ ID NO: 2 - protein, 469 aa, Pseudomonas nitroreducens
MSRYELLIDGRLQAAEHYDRVIDPASEEIVGEAARASLEQVDAAVDAAHRAFPAWATDLDVRRQSLARAAERVRENAQALAELITREQGRPLRSTLEEVAGVAATFEHHAQLELPADTQLRDDGERLVRITRKPLGVVAAITPWNVPLILLVLKIAPALHAGNTVVAKPSEHTPLSTLLLARLLGDVFPAGVFNVVAGAGEVGEHLVRHPRVRHVTFTGSVATGKRLYAGAGDDLKRLTLELGGNDAALVLEDADLDAIVEPLFWGAFWNSGQVCFAIKRLYVHDSLFEPLLAKLAERAQRTRLGHGLDPQTELGPLTNAQQLERVIALVEDAKAHGARIRSGGVRPDGPGYFYPPTLVSGVAAGVALVDEEQFGPVLPVISFRNEEDAITQANASHYGLGASVWTRDLARGEAIARRLEAGLAWVNQHGHIQPGAPKGGHKWSGLGYEGGQRGYEAFSELQVLNISRR

SEQ ID NO: 3 - DNA, 1437 bp, Saccharolobus solfataricus
  source 1..1437: mol_type = genomic DNA
atgaaatcgtatcagggattggctgacaagtggattaagggcagtggggaagaataccttgatattaatccggctgataaggatcacgtattagctaagataagattatatacaaaagatgacgttaaagaagctataaacaaggctgtagccaaattcgacgaatggtcaaggactccagcacctaaaagaggctcaatattacttaaggcaggggaattaatggaacaagaagcccaagagtttgcgctattgatgacattagaggagggtaagactctcaaggatagtatgtttgaagtgacaagaagttataatttactgaaattttatggagcattagcatttaagatatctgggaaaacgcttccttcagcagatcctaatactaggatatttacagtaaaggaacccttaggcgtagtagctttaattacgccgtggaatttcccattatcaataccagtatggaaattggctccagccttggctgcgggtaacactgcagtaataaaaccagcgacgaaaacaccgttaatggtagccaaattggtagaagtgttgtctaaagctggattgccagagggtgtcgtgaatttagtagttggtaagggaagtgaagtcggagataccatagtaagtgatgataatatagctgcagtatcatttactggatcaaccgaggtaggtaagagaatttacaaactcgtaggaaataaaaatagaatgacaagaattcaactagagctaggaggtaaaaacgcgttatatgtggataagagcgctgacttaacgttagctgctgaattagccgtaagaggaggatttggactaaccggtcaatcatgtactgcaactagtaggttaataattaacaaggatgtatatactcaatttaaacaaagactactagaaagagttaagaagtggagagtaggaccgggtactgaagatgttgatatgggtccagttgtagatgaaggtcaatttaagaaagacttagaatatatagaatacggaaagaatgtgggagcaaaactaatttatggtggaaatataataccagggaagggatatttcctagaacctacaattttcgaaggagtcacatctgatatgaggctatttaaagaagagattttcggtccagtacttagtgtcactgaggcaaaagatttagatgaggctataaggctagttaacgctgtagactatggacatacagctggaatagtcgcaagcgatatcaaggcgattaacgagttcgttagtagggtagaggcaggagttataaaggttaataagccaacagtcggactggaattgcaagcaccatttggtggttttaagaattctggagccactacgtggaaagagatgggagaagatgctttagagttctaccttaaggagaagacagtatacgaaggctggtaa

SEQ ID NO: 4 - protein, 478 aa, Saccharolobus solfataricus
MKSYQGLADKWIKGSGEEYLDINPADKDHVLAKIRLYTKDDVKEAINKAVAKFDEWSRTPAPKRGSILLKAGELMEQEAQEFALLMTLEEGKTLKDSMFEVTRSYNLLKFYGALAFKISGKTLPSADPNTRIFTVKEPLGVVALITPWNFPLSIPVWKLAPALAAGNTAVIKPATKTPLMVAKLVEVLSKAGLPEGVVNLVVGKGSEVGDTIVSDDNIAAVSFTGSTEVGKRIYKLVGNKNRMTRIQLELGGKNALYVDKSADLTLAAELAVRGGFGLTGQSCTATSRLIINKDVYTQFKQRLLERVKKWRVGPGTEDVDMGPVVDEGQFKKDLEYIEYGKNVGAKLIYGGNIIPGKGYFLEPTIFEGVTSDMRLFKEEIFGPVLSVTEAKDLDEAIRLVNAVDYGHTAGIVASDIKAINEFVSRVEAGVIKVNKPTVGLELQAPFGGFKNSGATTWKEMGEDALEFYLKEKTVYEGW

SEQ ID NO: 5 - DNA, 1410 bp, Methylovorus glucosotrophus
  source 1..1410: mol_type = genomic DNA
atgtcgacatttcatttacttattgatggccatctgcaagccagtgaccaatccgatgtggtgatcaaccccgcgaccgagctggaagtcgggcgtgccccacgtgccagcgccacccaggtcgaccaggcagtggaagccgcacatcaggcatttcatcgctgggcatcacagcctgaggtgcgccagcaggcactgctgggcgcggccgccgccattcgccagcatgccgatgccctggcacgcctgatcacgcaagagcaggggcggccattgcactttacccagggcgaggtggccggggctgctgctacctttgaacactatgccgggtttgccgcgccatcggatgtggtgctgcagcaggacgaacaaaagcgggtcagcattgagcgcaggccgtttggcgtagtggctgccattacgccctggaatgtgcccatcatcctgctggtactgaaaatcgccccggccttgaaggctggcaataccgtggtcgccaagccatcggaatacaccccgctttctaccttgtacctgggtgaaattctgaaagatgtatttccgcccggcgtgctgaacgtgatagccggtgacggtcaggtgggggcgcgcctggcatcgcatccgctggtgcagaaggtgacgttcaccggcagcgtggcaaccggaaaaaaactctatgccagcgccgcgcaggatgtaaaacgcctgacgctggaactgggcggtaacgatgcggccatcgtgctggacgatgccaatgtcgatgccattgccgagaagattttctggggcgccttctggaatagcggtcaggtgtgctttgccatcaagcgcctctatgtgcacgagcgtgttttccagcccttgctcgatgccctggtgaaacgcgcgcaaaaaacccgcgtgggcgatggccagctgccgggtaccgagctggggccgcttaccaacaaagcccagtttgagcgcgtgatatcgctggtggaagacgccagacgccatggcgccaccattcattcaggcggtgctgcattgcctggccccggctatttctatccgcccaccctggtcaccggcataggcgcaggtgtcgcgctggtggatgaagagcagttcggaccagtattgccgctgattcctttccgtgatgagcaagaggcggtgcgtcaggccaacgacagtccgtttggtctgggcgcttcggtttggaccgccaatcccgaacgcggcctggcgctggtacgccagctccaggccgggctcgcctgggtcaaccagcatggcgatatccatcccggtgcgcccaagggcggctacaaatccagtggccttggctacgagggcgggctgcgtggctatgacgagttcagcgagctgcaagtcgtcaatgcggcgctggtttaa

SEQ ID NO: 6 - protein, 469 aa, Methylovorus glucosotrophus
MSTFHLLIDGHLQASDQSDVVINPATELEVGRAPRASATQVDQAVEAAHQAFHRWASQPEVRQQALLGAAAAIRQHADALARLITQEQGRPLHFTQGEVAGAAATFEHYAGFAAPSDVVLQQDEQKRVSIERRPFGVVAAITPWNVPIILLVLKIAPALKAGNTVVAKPSEYTPLSTLYLGEILKDVFPPGVLNVIAGDGQVGARLASHPLVQKVTFTGSVATGKKLYASAAQDVKRLTLELGGNDAAIVLDDANVDAIAEKIFWGAFWNSGQVCFAIKRLYVHERVFQPLLDALVKRAQKTRVGDGQLPGTELGPLTNKAQFERVISLVEDARRHGATIHSGGAALPGPGYFYPPTLVTGIGAGVALVDEEQFGPVLPLIPFRDEQEAVRQANDSPFGLGASVWTANPERGLALVRQLQAGLAWVNQHGDIHPGAPKGGYKSSGLGYEGGLRGYDEFSELQVVNAALV

SEQ ID NO: 7 - DNA, 1062 bp, Galactocandida mastotermitis
  source 1..1062: mol_type = genomic DNA
atgagcacaccggaaaatctgagctttgtgctgcagaaaccgtttgatgtgaaatttgaagatcgtccgattccgaaactgagcgatccgtatagcgttaaaattcaggtgaaaaaaaccggcatttgcggtagtgatgttcactatttcacccatggtgcaattggtgattttgttgttaaagcaccgatggttctgggtcatgaaagcagcggtgttgttctggaagttggtagcgaagttaaaagcctgaaagttggtgatcgtgttgcaatggaaccgggtgttccgagccgtcatagtgatgagtataaaagcggtcgttataatctgtgtccgcacatggcatttgcagcaacccctccgtatgatggcaccctgtgtaaatactatattctgccggaagatttctgcgttaaactgccggaacatgttagcctggaagaaggtgcactggttgaaccgctgagcgttgcagttcatagcagcaaactgggtaacattaaaccgggtagccatgttgcaatttatggtgcaggtccggttggtctgctggttgcagcagttgcaagcgcatttggtgcagaaagcgttaccattattgatctggttgaaagccgtctgaatctggcaaaagaactgggtgcaaccgcaaccgttcaggttgattttaaagataccccgaaagaaagcgcagcaaaagttgttgcagcaaataatggcattgcaccggatgttgttattgatgcaagcggtgcagaagcaagcattaattcagccattaatgcaattcgtccgggtggcacctatgttcaggtgggtatgggtaaaccggatgtgagctttccgattgcaaccctgattggtaaagaactgaccgttaaaggtagctttcgttatggttatggtgattatccgctggcagttagcctgctggcaagcggtaaagttaatgtgaaaaaactgatcacccatgaagtgaaattcgaggatgcagcagaagcatttcagctggttcgtgatggtaaagccattaaatgtattatcaacggtccggaataa

SEQ ID NO: 8 - protein, 353 aa, Galactocandida mastotermitis
MSTPENLSFVLQKPFDVKFEDRPIPKLSDPYSVKIQVKKTGICGSDVHYFTHGAIGDFVVKAPMVLGHESSGVVLEVGSEVKSLKVGDRVAMEPGVPSRHSDEYKSGRYNLCPHMAFAATPPYDGTLCKYYILPEDFCVKLPEHVSLEEGALVEPLSVAVHSSKLGNIKPGSHVAIYGAGPVGLLVAAVASAFGAESVTIIDLVESRLNLAKELGATATVQVDFKDTPKESAAKVVAANNGIAPDVVIDASGAEASINSAINAIRPGGTYVQVGMGKPDVSFPIATLIGKELTVKGSFRYGYGDYPLAVSLLASGKVNVKKLITHEVKFEDAAEAFQLVRDGKAIKCIINGPE

SEQ ID NO: 9 - DNA, 1014 bp, Geobacillus stearothermophilus
  source 1..1014: mol_type = genomic DNA
atgaaagctgcagttgtggaacaatttaaaaagccgttacaagtgaaagaagtggaaaaacctaagatctcatacggggaagtattagtgcgcatcaaagcgtgtggggtatgccatacagacttgcatgccgcacatggcgactggcctgtaaagcctaaactgcctctcattcctggccatgaaggcgtcggtgtaattgaagaagtaggtcctggggtaacacatttaaaagttggagatcgcgtaggtatcccttggctttattcggcgtgcggtcattgtgactattgcttaagcggacaagaaacattatgcgaacgtcaacaaaacgctggctattccgtcgatggtggttatgctgaatattgccgtgctgcagccgattatgtcgtaaaaattcctgataacttatcgtttgaagaagccgctccaatcttttgcgctggtgtaacaacatataaagcgctcaaagtaacaggcgcaaaaccaggtgaatgggtagccatttacggtatcggcgggcttggacatgtcgcagtccaatacgcaaaggcgatggggttaaacgtcgttgctgtcgatttaggtgatgaaaaacttgagcttgctaaacaacttggtgcagatcttgtcgtcaatccgaaacatgatgatgcagcacaatggataaaagaaaaagtgggcggtgtgcatgcgactgtcgtcacagctgtttcaaaagccgcgttcgaatcagcctacaaatccattcgtcgcggtggtgcttgcgtactcgtcggattaccgccggaagaaatacctattccaattttcgatacagtattaaatggagtaaaaattattggttctatcgttggtacgcgcaaagacttacaagaggcacttcaatttgcagcagaaggaaaagtaaaaacaattgtcgaagtgcaaccgcttgaaaacattaacgacgtattcgatcgtatgttaaaagggcaaattaacggccgcgtcgtgttaaaagtagattaa

SEQ ID NO: 10 - protein, 337 aa, Geobacillus stearothermophilus
MKAAVVEQFKKPLQVKEVEKPKISYGEVLVRIKACGVCHTDLHAAHGDWPVKPKLPLIPGHEGVGVIEEVGPGVTHLKVGDRVGIPWLYSACGHCDYCLSGQETLCERQQNAGYSVDGGYAEYCRAAADYVVKIPDNLSFEEAAPIFCAGVTTYKALKVTGAKPGEWVAIYGIGGLGHVAVQYAKAMGLNVVAVDLGDEKLELAKQLGADLVVNPKHDDAAQWIKEKVGGVHATVVTAVSKAAFESAYKSIRRGGACVLVGLPPEEIPIPIFDTVLNGVKIIGSIVGTRKDLQEALQFAAEGKVKTIVEVQPLENINDVFDRMLKGQINGRVVLKVD